European Patent Application EP 4 541 904 A1, published April 23, 2025. Title: SEQUENCING KIT CONTAINING SULFYDRYL BLOCKING REAGENT AND APPLICATION OF SEQUENCING KIT. Applicant: MGI Tech Co., Ltd. The sequence listing filed with the application follows.

SEQUENCE LISTING (1 sequence)

SEQ ID NO: 1 - DNA, 39 bp, synthetic construct
  source 1..39: mol_type = other DNA
caactccttggctcacagaacatggctacgatccgactt